European Patent Application EP 4 582 552 A1, published July 9, 2025. Title: Differential Methylation Region of OPLAH Gene, Kit, and Use. Applicant: BGI GENOMICS CO., LTD. Application WO PCT/CN2022/116734, filed September 2, 2022. The sequence listing filed with the application follows.

SEQUENCE LISTING (110 sequences)

SEQ ID NO: 1 - DNA, 1297 bp, Homo sapiens
  source 1..1297: mol_type = genomic DNA
cgccgtagctgcgtccccagaaccgggagacttaaggcatctttattgcgggatcctcacacggcctcctgggcccggcgatactcatagacgctgccgtgctcgggaaaggccagtgcttgcgggggcgaccccggcggtggggcggggtcctccgggtccccatagccaccgccgccgggcgtgtggagacagaacacatcctgttggcgcgggggggggcggggaggcgggctcagtgcaggcgtggcccctccctgtcacctgcgcagtcccctccccaccgggcagcgtccatcacccgcccccatggaccacggaggcccggtacgcgccccctttccttccggggccaaattaaactcggcctctggtcaggtctgcaactgttccccctctgtgggatggggccgggaggggaggggaggggagggggacaggacaggccgcggcccttaccccggggtacacggtcaccgacgtcttgccgcccagattcaccgtccggccgtttttgcggatcagcaggtttaggccgcgggcgccaggctcgccccctgcggagggaggcgaggagtccagagagaccaggggcgggggtgggggcgggggcggggagggccgcgagggctggggaaccgcgcaccgtggagcccgtatggccggaaggcgcggcgctcggtcagcactgacagcagcgcctcctcacgaaagagcagctcgcgggtgacgccgtcgccgcctcggaagcggcctctgccccccgagccccccgccgcagctcgaagcggcgcaggatgaccgggtacctgcgagggcgaggacgagggcaaagactcagcgtggcccgagccccggctcccacccggccgtgcccccagcctccgcgcacgccgctcaccggctctccaggatctcagggtcggtgatgcgtgtgttggtcatgtggctgtgcacaccgctgcgcccgtgccagctgggacccgcgcccgcgccgcccgccaccgtctcgtagtagcccatgtgggcgttgcccagggtcacgttgttcatgcagccctggtgagggcacctggtcgctgcgctgggctggggcagggcgtccccacctcgccctcccgctcctactccagcctgcccacccagtccgcccccgagctgcgcccaccccgcccccgcacctgggaggcggcgcaggccccaaaggcccccaggatgacatccaccacgcgctgcgacgtgagcacgttgccgcccaccaccgccgcctcgggcgacgggtccaggatggagcctc

SEQ ID NO: 2 - DNA, 20 bp, synthetic construct
  source 1..20: mol_type = other DNA
gaattaggcgtcgtagttgc

SEQ ID NO: 3 - DNA, 20 bp, synthetic construct
  source 1..20: mol_type = other DNA
cgcaaacactaacctttccc

SEQ ID NO: 4 - DNA, 22 bp, synthetic construct
  source 1..22: mol_type = other DNA
gggttcggcgatatttatagac

SEQ ID NO: 5 - DNA, 16 bp, synthetic construct
  source 1..16: mol_type = other DNA
ccccaccgccgaaatc

SEQ ID NO: 6 - DNA, 24 bp, synthetic construct
  source 1..24: mol_type = other DNA
agtacggtagcgtttatgagtatc

SEQ ID NO: 7 - DNA, 20 bp, synthetic construct
  source 1..20: mol_type = other DNA
aactaaacgccgtaactacg

SEQ ID NO: 8 - DNA, 20 bp, synthetic construct
  source 1..20: mol_type = other DNA
ttatcgtcggggtcgttttc

SEQ ID NO: 9 - DNA, 26 bp, synthetic construct
  source 1..26: mol_type = other DNA
acatctttattacgaaatcctcacac

SEQ ID NO: 10 - DNA, 19 bp, synthetic construct
  source 1..19: mol_type = other DNA
tcgtcgggtttaggaggtc

SEQ ID NO: 11 - DNA, 21 bp, synthetic construct
  source 1..21: mol_type = other DNA
actcgaaacacgaactaaacg

SEQ ID NO: 12 - DNA, 25 bp, synthetic construct
  source 1..25: mol_type = other DNA
tatttttattgcgggatttttatac

SEQ ID NO: 13 - DNA, 25 bp, synthetic construct
  source 1..25: mol_type = other DNA
caaaatatattctatctccacacgc

SEQ ID NO: 14 - DNA, 22 bp, synthetic construct
  source 1..22: mol_type = other DNA
cgtagttgcgtttttagaatcg

SEQ ID NO: 15 - DNA, 22 bp, synthetic construct
  source 1..22: mol_type = other DNA
tataaaaacccgaaaaaccccg

SEQ ID NO: 16 - DNA, 21 bp, synthetic construct
  source 1..21: mol_type = other DNA
gggtagtgcgtttgtagtttc

SEQ ID NO: 17 - DNA, 22 bp, synthetic construct
  source 1..22: mol_type = other DNA
cgacaacgtctataaatatcgc

SEQ ID NO: 18 - DNA, 24 bp, synthetic construct
  source 1..24: mol_type = other DNA
ttttggaggggtttacggattatc

SEQ ID NO: 19 - DNA, 24 bp, synthetic construct
  source 1..24: mol_type = other DNA
ccaaaaaaccgtataaaaatcccg

SEQ ID NO: 20 - DNA, 23 bp, synthetic construct
  source 1..23: mol_type = other DNA
aaggtaagtatagatgaggggcg

SEQ ID NO: 21 - DNA, 21 bp, synthetic construct
  source 1..21: mol_type = other DNA
cgcaaacactaacctttcccg

SEQ ID NO: 22 - DNA, 20 bp, synthetic construct
  source 1..20: mol_type = other DNA
gaggtcgtgtgaggatttcg

SEQ ID NO: 23 - DNA, 21 bp, synthetic construct
  source 1..21: mol_type = other DNA
aacaatacgcctacaactccg

SEQ ID NO: 24 - DNA, 22 bp, synthetic construct
  source 1..22: mol_type = other DNA
gggtagtgcgtttgtagtttcg

SEQ ID NO: 25 - DNA, 25 bp, synthetic construct
  source 1..25: mol_type = other DNA
acacgacaacgtctataaatatcgc

SEQ ID NO: 26 - DNA, 23 bp, synthetic construct
  source 1..23: mol_type = other DNA
tcgggtagtgcgtttgtagtttc

SEQ ID NO: 27 - DNA, 24 bp, synthetic construct
  source 1..24: mol_type = other DNA
ggtttacggattatcgggtagtgc

SEQ ID NO: 28 - DNA, 24 bp, synthetic construct
  source 1..24: mol_type = other DNA
cgacaacgtctataaatatcgccg

SEQ ID NO: 29 - DNA, 19 bp, synthetic construct
  source 1..19: mol_type = other DNA
gggcgttgtttagggttac

SEQ ID NO: 30 - DNA, 18 bp, synthetic construct
  source 1..18: mol_type = other DNA
aaacgcaactcgaaaacg

SEQ ID NO: 31 - DNA, 17 bp, synthetic construct
  source 1..17: mol_type = other DNA
ccctaccccaacccaac

SEQ ID NO: 32 - DNA, 21 bp, synthetic construct
  source 1..21: mol_type = other DNA
cgttcgtgttagttgggattc

SEQ ID NO: 33 - DNA, 25 bp, synthetic construct
  source 1..25: mol_type = other DNA
cataaacaacgtaaccctaaacaac

SEQ ID NO: 34 - DNA, 23 bp, synthetic construct
  source 1..23: mol_type = other DNA
gggacgttttgttttagtttagc

SEQ ID NO: 35 - DNA, 19 bp, synthetic construct
  source 1..19: mol_type = other DNA
cccgtaccaactaaaaccc

SEQ ID NO: 36 - DNA, 19 bp, synthetic construct
  source 1..19: mol_type = other DNA
tatttgcgagggcgaggac

SEQ ID NO: 37 - DNA, 22 bp, synthetic construct
  source 1..22: mol_type = other DNA
cctaaaaaaccgataaacgacg

SEQ ID NO: 38 - DNA, 21 bp, synthetic construct
  source 1..21: mol_type = other DNA
cgttcgtgttagttgggatgc

SEQ ID NO: 39 - DNA, 24 bp, synthetic construct
  source 1..24: mol_type = other DNA
taaacaacgtaaccctaaacaccg

SEQ ID NO: 40 - DNA, 19 bp, synthetic construct
  source 1..19: mol_type = other DNA
gggcgttgtttagggttgc

SEQ ID NO: 41 - DNA, 17 bp, synthetic construct
  source 1..17: mol_type = other DNA
cctaccccaacccaccg

SEQ ID NO: 42 - DNA, 21 bp, synthetic construct
  source 1..21: mol_type = other DNA
cgttcgtgttagttgggcttc

SEQ ID NO: 43 - DNA, 24 bp, synthetic construct
  source 1..24: mol_type = other DNA
taaacaacgtaaccctaaaccacg

SEQ ID NO: 44 - DNA, 21 bp, synthetic construct
  source 1..21: mol_type = other DNA
cgttcgtgttagttgggatcc

SEQ ID NO: 45 - DNA, 21 bp, synthetic construct
  source 1..21: mol_type = other DNA
cgttcgtgttagttggggttc

SEQ ID NO: 46 - DNA, 24 bp, synthetic construct
  source 1..24: mol_type = other DNA
taaacaacgtaaccctaaacgacg

SEQ ID NO: 47 - DNA, 24 bp, synthetic construct
  source 1..24: mol_type = other DNA
taaacaacgtaaccctaaacaacg

SEQ ID NO: 48 - DNA, 17 bp, synthetic construct
  source 1..17: mol_type = other DNA
cctaccccaacccaacg

SEQ ID NO: 49 - DNA, 18 bp, synthetic construct
  source 1..18: mol_type = other DNA
aagcggcgtaggatgatc

SEQ ID NO: 50 - DNA, 17 bp, synthetic construct
  source 1..17: mol_type = other DNA
ccgaaactcgaaccacg

SEQ ID NO: 51 - DNA, 19 bp, synthetic construct
  source 1..19: mol_type = other DNA
aaaccgaaactcgaaccac

SEQ ID NO: 52 - DNA, 19 bp, synthetic construct
  source 1..19: mol_type = other DNA
tttaaaacctacgccgcct

SEQ ID NO: 53 - DNA, 21 bp, synthetic construct
  source 1..21: mol_type = other DNA
acgaaataaaaacgccctacc

SEQ ID NO: 54 - DNA, 28 bp, synthetic construct
  source 1..28: mol_type = other DNA
actcgaaaacgaactaaataaacaaact

SEQ ID NO: 55 - DNA, 24 bp, synthetic construct
  source 1..24: mol_type = other DNA
tgaataacgtgattttgggtaacg

SEQ ID NO: 56 - DNA, 24 bp, synthetic construct
  source 1..24: mol_type = other DNA
cgactctccaaaatctcaaaatcg

SEQ ID NO: 57 - DNA, 22 bp, synthetic construct
  source 1..22: mol_type = other DNA
gggtaaagatttagcgtggttc

SEQ ID NO: 58 - DNA, 19 bp, synthetic construct
  source 1..19: mol_type = other DNA
acgaaataaacgcaactcg

SEQ ID NO: 59 - DNA, 19 bp, synthetic construct
  source 1..19: mol_type = other DNA
cgcaactcgaaaacgaact

SEQ ID NO: 60 - DNA, 20 bp, synthetic construct
  source 1..20: mol_type = other DNA
aggatgatcgggtatttgcg

SEQ ID NO: 61 - DNA, 21 bp, synthetic construct
  source 1..21: mol_type = other DNA
caaccacataaccaacacacg

SEQ ID NO: 62 - DNA, 19 bp, synthetic construct
  source 1..19: mol_type = other DNA
gcgaatcccaactaacacg

SEQ ID NO: 63 - DNA, 21 bp, synthetic construct
  source 1..21: mol_type = other DNA
gacgagggtaaagatttagcg

SEQ ID NO: 64 - DNA, 22 bp, synthetic construct
  source 1..22: mol_type = other DNA
ggtaaagatttagcgtggttcg

SEQ ID NO: 65 - DNA, 25 bp, synthetic construct
  source 1..25: mol_type = other DNA
tcggttttttaggattttagggtcg

SEQ ID NO: 66 - DNA, 25 bp, synthetic construct
  source 1..25: mol_type = other DNA
cctcaccaaaactacataaacaacg

SEQ ID NO: 67 - DNA, 29 bp, synthetic construct
  source 1..29: mol_type = other DNA
ttgtatgaataacgtgattttgggtaacg

SEQ ID NO: 68 - DNA, 27 bp, synthetic construct
  source 1..27: mol_type = other DNA
caccgactctccaaaatctcaaaatcg

SEQ ID NO: 69 - DNA, 28 bp, synthetic construct
  source 1..28: mol_type = other DNA
ttatcgattttgagattttggagagtcg

SEQ ID NO: 70 - DNA, 23 bp, synthetic construct
  source 1..23: mol_type = other DNA
ctcgatcaacactaacaacaacg

SEQ ID NO: 71 - DNA, 23 bp, synthetic construct
  source 1..23: mol_type = other DNA
gcgtaggatgatcgggtatttgc

SEQ ID NO: 72 - DNA, 22 bp, synthetic construct
  source 1..22: mol_type = other DNA
cgaatcccaactaacacgaacg

SEQ ID NO: 73 - DNA, 16 bp, synthetic construct
  source 1..16: mol_type = other DNA
tttgcggagggaggcg

SEQ ID NO: 74 - DNA, 18 bp, synthetic construct
  source 1..18: mol_type = other DNA
gcgattccccaaccctcg

SEQ ID NO: 75 - DNA, 23 bp, synthetic construct
  source 1..23: mol_type = other DNA
ggagtttagagagattaggggcg

SEQ ID NO: 76 - DNA, 19 bp, synthetic construct
  source 1..19: mol_type = other DNA
cgaccatacgaactccacg

SEQ ID NO: 77 - DNA, 20 bp, synthetic construct
  source 1..20: mol_type = other DNA
tcgtggagttcgtatggtcg

SEQ ID NO: 78 - DNA, 19 bp, synthetic construct
  source 1..19: mol_type = other DNA
cccgcgaactactctttcg

SEQ ID NO: 79 - DNA, 31 bp, synthetic construct
  source 1..31: mol_type = other DNA
acacgacaacgtctataaatatcgccgaacc

SEQ ID NO: 80 - DNA, 28 bp, synthetic construct
  source 1..28: mol_type = other DNA
cccgacgatactcataaacgctaccgta

SEQ ID NO: 81 - DNA, 26 bp, synthetic construct
  source 1..26: mol_type = other DNA
ccgtaactacgtccccaaaaccgaaa

SEQ ID NO: 82 - DNA, 24 bp, synthetic construct
  source 1..24: mol_type = other DNA
tcgggtttaggaggtcgtgtgagg

SEQ ID NO: 83 - DNA, 24 bp, synthetic construct
  source 1..24: mol_type = other DNA
aaccgtataaaaatcccgcaataa

SEQ ID NO: 84 - DNA, 28 bp, synthetic construct
  source 1..28: mol_type = other DNA
aaacgcaactacgacgcctaattcgtac

SEQ ID NO: 85 - DNA, 27 bp, synthetic construct
  source 1..27: mol_type = other DNA
ttggcgcgtatagatacgattcggagt

SEQ ID NO: 86 - DNA, 22 bp, synthetic construct
  source 1..22: mol_type = other DNA
tagtgcgtttgtagtttcgagt

SEQ ID NO: 87 - DNA, 21 bp, synthetic construct
  source 1..21: mol_type = other DNA
ctcccgattctaaaaacgcaa

SEQ ID NO: 88 - DNA, 17 bp, synthetic construct
  source 1..17: mol_type = other DNA
acgtagttacggcgttt

SEQ ID NO: 89 - DNA, 19 bp, synthetic construct
  source 1..19: mol_type = other DNA
caacgaccaaataccctca

SEQ ID NO: 90 - DNA, 22 bp, synthetic construct
  source 1..22: mol_type = other DNA
ttcgcgtcgttcgttatcgttt

SEQ ID NO: 91 - DNA, 22 bp, synthetic construct
  source 1..22: mol_type = other DNA
agcgtggttcgagtttcggttt

SEQ ID NO: 92 - DNA, 23 bp, synthetic construct
  source 1..23: mol_type = other DNA
atttggtcgttgcgttgggttgg

SEQ ID NO: 93 - DNA, 19 bp, synthetic construct
  source 1..19: mol_type = other DNA
cccgccaccgtctcgtaat

SEQ ID NO: 94 - DNA, 20 bp, synthetic construct
  source 1..20: mol_type = other DNA
ttgcgagggcgaggacgagg

SEQ ID NO: 95 - DNA, 26 bp, synthetic construct
  source 1..26: mol_type = other DNA
cgaggacgagggtaaagatttagcgt

SEQ ID NO: 96 - DNA, 32 bp, synthetic construct
  source 1..32: mol_type = other DNA
aacgcaacgatatacacaaccacataaccaac

SEQ ID NO: 97 - DNA, 29 bp, synthetic construct
  source 1..29: mol_type = other DNA
ttcgagtttcggtttttattcggtcgtgt

SEQ ID NO: 98 - DNA, 21 bp, synthetic construct
  source 1..21: mol_type = other DNA
ttcggtttttattcggtcgtg

SEQ ID NO: 99 - DNA, 29 bp, synthetic construct
  source 1..29: mol_type = other DNA
caccgaccctaaaatcctaaaaaaccgat

SEQ ID NO: 100 - DNA, 26 bp, synthetic construct
  source 1..26: mol_type = other DNA
accgataaacgacgtacgcgaaaact

SEQ ID NO: 101 - DNA, 27 bp, synthetic construct
  source 1..27: mol_type = other DNA
ctacgaaacgataacgaacgacgcgaa

SEQ ID NO: 102 - DNA, 21 bp, synthetic construct
  source 1..21: mol_type = other DNA
acgagggtaaagatttagcgt

SEQ ID NO: 103 - DNA, 22 bp, synthetic construct
  source 1..22: mol_type = other DNA
cacaccgctacgcccgtaccaa

SEQ ID NO: 104 - DNA, 18 bp, synthetic construct
  source 1..18: mol_type = other DNA
tgagcggcgtgcgcggag

SEQ ID NO: 105 - DNA, 21 bp, synthetic construct
  source 1..21: mol_type = other DNA
agtttagagagattaggggcg

SEQ ID NO: 106 - DNA, 25 bp, synthetic construct
  source 1..25: mol_type = other DNA
tacgcgattccccaaccctcgcgac

SEQ ID NO: 107 - DNA, 20 bp, synthetic construct
  source 1..20: mol_type = other DNA
aaggcgcggcgttcggttag

SEQ ID NO: 108 - DNA, 23 bp, synthetic construct
  source 1..23: mol_type = other DNA
tttaggagtgagtggaagataga

SEQ ID NO: 109 - DNA, 23 bp, synthetic construct
  source 1..23: mol_type = other DNA
aaaccacaccatcctaattacct

SEQ ID NO: 110 - DNA, 23 bp, synthetic construct
  source 1..23: mol_type = other DNA
cccaaaacacatttcttccattc